European Patent Specification EP 3 782 628 B1, published August 7, 2024. Title: METHODS OF USING ZSCAN4 FOR REJUVINATING HUMAN CELLS. Applicant: Ko, Minoru S.H. Application Not Yet Assigned. The sequence listing filed with the application follows.

SEQUENCE LISTING (44 sequences)

SEQ ID NO: 1 - DNA, 2275 bp, Mus musculus
cacagtgcctccctgggcttcttggcatcacccttgaagttcactggagaaagagttgaggtggaggaataggtaaacttcccttcctagtggtcttgaatgtcttttacagtacatccatcaactgttagcattttcgtaaagtcacaaaacagatattaaactactatagttgaatctttcacaccattgtcaccacaatggcttcacagcaggcaccagcaaaagaccttcagaccaacaatttagagtttactccaactgatagttctggtgtgcagtgggcagaagacatctctaactcaccaagtgctcagctaaacttttccccaagtaacaatggctgctgggcaactcaggagctgcaaagtctctggaagatgttcaactcctggttgcagccagaaaagcagactaaggagcagatgatttctcaactggtcttggagcagtttctcctcactgggcactgcaaggacaagtatgctttgacagagaagtggaaagccagtggtagcgatatgaggagattcatggagagtctgactgatgagtgcttgaagcctcctgtcatggtccatgtctcaatgcaaggacaagaagccctcttttctgaaaacatgccattaaaagaagtcatcaagcttttgaaacaacagcaatctgcaacaaggccaacaccagataatgcacagatgccagtagacaccacacaagatagattattggccacaggacaagaaaacagtgaaaatgaatgcaacacctcttgtaatgctactgaaggaaatgttggtgagagctgtagtggaaatgaaatggactcctctcttattatccagaaagaacagtaccctgagcatgaagaggggaatgttgtttgtcaattccctcttgatgccagaagagcaagtcaaggcacctccagtcatcatgtagacttcctgagtgctctgactactgccgatgtccccatggaggaacaaccaaaggatttatccagagaaaacatctctgaggacaagaacaattgctataacacttccaggaatgcagctactaaagtatatagtggtgataatattcccaggaaaaagacagactccctttccattaacaagaggatatatcatcctgagcctgaggtgggagatattccttatggagttcctcaggattctacaagagcaagtcaaggaacatctacatgcctgcaagagtcacttgggggatgtttttccgaaaaagaccctagggaggtaccagggttgcagtctaggtaagagcagcctatctctgatcctgtccttcttggtaagaatcatgaggcaaacttaccatgtgaaagtcatcaaaagagattctgtagagatgccaaactatacaagtgtgaagaatgttctaggatgttcaaacatgccaggagcctttcatcccaccagagaactcacctgaataagaagagtgaattgctttgtgtcacctgtcagaaaattttcaaacgagtctctgaccgccgaacccatgagatcatacacatgccagaaaagcctttcaagtgcagcacatgtgaaaagtccttcagccacaagaccaacctgaagtctcatgagatgattcacacaggagaaatgccttatgtctgttccctatgtagccgtcgctttcgccaatcatccacttaccatcgtcacctgaggaattatcacagatctgactgaagtatctaacatcctcagcagagactggtagggcttcagcctcagtatgtcatcttcaaagagagaagaatgttgcaagtaaattgtactgtcccaataatgatataacatgcttgtggattgccacttttatgttttgttttgttttgttttttattttgtgtgtgtgtatgtaattttttgtctgtatttccatagttccacagcataagttattagaatactttgctgttaattcttgagttgcttcttgcttttagacagtgtctttctggttggcagctttatacacctgtctttctggcactagagtttccaaacattttctgatctccacttttattttctacagtggtcctgacagaggcctgccattccctctgacatttttctacatgttggggtttcatcccaagtcttagggttgcaagttaaatgcattgcctcttcagacatctcatgtcatgtctactgcttacagttcaagaatatttctctacattactagaacgacgttcaaagtggaataataaataaataaataatcaacaatt

SEQ ID NO: 2 - DNA, 1774 bp, Mus musculus
cacagtgcctccctgggcttcttggcatcacccttgaagttcactggagaaagaggtgatgtggagaagtaggtaaacttccctttcttgtggtcttgaatgtcttttacagtacatccgtcaactgttagcattttcctaaagtcacaaaacagatactaaactgctatagttgaatctttcagaccattgtcaccacaatggcttcacagcaggcaccagcaaaagaccttcagaccaacaatttagagtttactccaactgatagttctggtgtgcagtgggcagaagacatctctaactcaccaagtgctcagctaaacttttccccaagtaacaatggctgctgggcaactcaggagctgcaaagtctctggaagatgttcaactcctggttgcagccagaaaagcagactaaggagcagatgatttctcaattggtcttggagcagtttctcctcactgggcactgcaaggacaagtatgctttgacagagaagtggaaagccagtggtagcgatatgaggagattcatggagagtctgactgatgagtgcttgaagcctcctgtcatggtccatgtttcaatgcaaggacaagaagccctcttttctgaaaacatgccattaaaagaagtcatcaagcttttgaaacaacagcaatctgcaacaaggccaataccagataatgcacagatgccagtagacaccacacaagatagattattggccacaggcaagaaaacagtgaaaatgaatgcaacacctcttgcaatgctactgaagtaaatgttggtgaaagctgtagtggaaatgaaaaggactcccttcttattacccagaaagaacaaaaccatgagcatgaagaggggaatgttgtttgtcaattccctcgtggtgccagaagagcaagtcaagacacctccagtcatcatgtagacttcccgagtgctctgactcctgcagatgtccccatggaggaacaaccaatggatttatccagagaaaacatctctgaggacaagaacaattgctataacacttccaggaatgcagctactcaagtatatagtggtgataatattcccaggaacaagacagactcccttttcattaacaagagaatatatcatcctgagcctgaggtgggagatattccttatggagttcctcaggattctacaagagcaagtcaaggaacatctacatgcctgcaagagtcacttggggaatgtttttctgaaaaagacccaagggaggtaccagggttgcagtctaggcaagagcagcctatctctgatcctgtccttggtaagaatcatgaggcaaacttaccatgtgaaagtcatcaaaagagattccatagagatgccaaactatacaagtgtgaagaatgttctaggatgttcaaacatgccaggagcctttcatcccaccagagaactcacctgaataagaagagtgaattgctttgcatcacctgtcagaaaatattcaaacgagtttctgaccttcgaacccatgagatcatacacatgtcagaaaagcctttcaagtgcagcacatgtgaaaagtccttcagccacaagaccaacctgaagtatcatgagatgattcacacaggagaaatgccttatgtctgttccctatgtagccgtcgctttcgccaatcatccacttaccatcgtcacctgaggaattaccacagatctgactgaagtatctaacatcctcagcagagactggtagggcttcagcctcagtatgtcatcttc

SEQ ID NO: 3 - DNA, 2275 bp, Mus musculus
cacagtgcctccctgggcttcttggcatcacccttgaagttcaccggagaaagcagtgaggtggaggaataggtaaactttccttcctagtggtcttgaatgtcttttacagtacatccatcaactgttagcattttcgtaaagtcacaaaacagatattaaactactatagttgaatctttcacaccattgtcaccacaatggcttcacagcaggcaccagcaaaagaccttcagaccaacaatttagagtttactccaactgatagttctggtgtgcagtgggcagaagacatctctaactcaccaagtgctcagctaaacttttccccaagtaacaatggctgctgggcaactcaggagctgcaaagtctctggaagatgttcaactcctggttgcagccagaaaagcagactaaggagcagatgatttctcaactggtcttggagcagtttctcctcactgggcactgcaaggacaagtatgctttgacagagaagtggaaagccagtggtagcgatatgaggagattcatggagagtctgactgatgagtgcttgaagcctcctgtcatggtccatgtttcaatgcaaggacaagaagccctcttttctgaaaacatgccattaaaagaagtcatcaagcttttgaaacaacagcaatctgcaacaaggccaacaccagataatgagcagatgccagtagacaccacacaagatagattattggccacaggacaagaaaacagtgaaaatgaatgcaacaactcttgtaatgctactgaagcaaatgttggtgaaagctgtagtggaaatgaaatggactcccttcttattatccagaaagaacagcaccctgagcatgaagaggggaatgttgtttgtcaattccctcatggtgccagaagagcaagtcaaggcacccccagtcatcatgtagacttcccgagtgctccgactactgccgatgtccccatggaggaacaaccaaaggatttatccagagaaaacatctctgaggacaagaacaattgctataacacttccagaaatgcagctactcaagtatatagtggtgataatattcccaggaacaagtcagactcccttttcattaacaagagaatatatcatcctgagcctgaggtgggagatattccttatggagttcctcaggattctacaagagcaagtcaaggaacatctacatgcctgcaagagtcacttggggaatgtttttctgaaaacgacccaagggaggtaccagggttgcagtctaggcaagagcagcctatctctgatcctgtccttcttggtaagaatcatgaggcaaacttaccatgtgaaagtcatcaaaagagattctgtagagatgccaaactatacaagtgtgaagaatgttctaggatgttcaaacatgccaggagcctttcatcccaccagagaactcacctgaataagaagagtgaattgctttgtgtcacctgtcagaaaatgttcaaacgagtctctgaccgccgaacccatgagatcatacacatgccagaaaagcctttcaagtgcagcacatgtgaaaagtccttcagccacaagaccaacctgaagtctcatgagatgattcacacaggagaaatgccttatgtctgttccctatgtagccgtcgctttcgccaatcatccacttaccatcgtcacctgaggaattaccacagatctgactgaactatctaacatcctcagcagagactggtagggcttcagcctcagtatgtcatcttcaaagagagaagaatgttgcaagtaaattgtactgtcccaataatgatataacatgcttgtggattgccacttttatgttttgttttgttttgttwtttatkttgtgtgtgtgtatgtaattttttgtctgtatttccatatttccacagcataagttattagaatactttgctgttaattcttgagttgcttcttgcttttagacagtgtctttctggttggcagctttatacacctgtctttctggcactagagtttccaaacattttctgatctccacttttattttctacagtgttcttgacagaagcctggcattccctctgacattttctacatgttggggttttcatcccaagtcttagggttgcaagttaaatgcattgcctcttcagacatctcatgccatgtctactgcttacagttcaagaatatttctctacattactagaacgacgttcaaagtggaataataaataaataaataatcaacaatt

SEQ ID NO: 4 - DNA, 2268 bp, Mus musculus
cacagtgcctccctgggcttcttggcatcacccttgaagttcactggacaaagaggtgaggtggaggagtaggtaaacttcccttcctagtggtcgtgaatgtcttttacagtacatccatcaactgttagcattttcataaagtcacaaaacagatactaaactgctatagttgaatctttcacaccattgtcaccacaatggcttcacagcaggcaccagcaaaagaccttcagaccaacaatttagagtttactccatctcatagttctggtgtgcagtgggtagaagacatctctaactcaccaagtgctcagctaaacttttctccaagtaacaatggctgctgggcaactcaggagctgcaaagtctctggaagatgttcaactcctggttgcagccagaaaagcagactaaggagcagatgatttctcaactggtcttggagcagtttctcctcattgggcactgcaaggacaagtatgctttgacagagaagtggaaagccagtggtagcgatatgaggagattcatggagagtctgactgatgagtgcttgaagcctcctgtcatggtccatgtttcaatgcaaggacaagaagctctcttttctgaaaacatgccattaaaagaagtcatcaagcttttgaaacaacagcaatctgcaacaaggccaacaccagataatgagcagatgccagtagacaccacacaagatagattattggccacaggacaagaaaacagtgaaaatgaatgcaacaactcttgtaatgctactgaagcaaatgttggtgaaagctgtagtggaaatgaaatggactcccttcttattatccagaaagaacagcaccctgagcatgaagaggggaatgttgtttttcaattccctcttgatgccagaagagcaagtcaaggcaactccagtcatcatgtagacttccggagtgctccgactcctgcggatgtccccatggaggaacaaccaaaggatttatccagagaaaacatctctgaggacaagaacaattgctataacacttccaggaatgcagctactcaagtatatagaagtgataatattcccaggaaaaagacagactccctttccattaacaagagaatatatcattctgagcctgaggagggagatattccttatggagttcctcaggattctacaagagcaagtcaaggaacatctacatgcttgcaagagtcacttggggaatgtttttctgaaaaagaccctagggagctaccagggttggagtctaggcaagaggagcctatctctgatcctgtctttcttggtaaggatcatgaggcaaacttaccatgtgaaagtcatcaaaagagattccgtagagatgccaaactattcaagtgtgaagaatgttctaggatgttcaaacatgccaggagcctttcgtcccaccagagaactcacctgaataagaagagtgaattgctttgtgtcacctgtcagaaaatgttcaaacgagtctctgaccgccgaacccatgagatcatacacatgccagaaaagcctttcaagtgcagcacatgtgaaaagtccttcagccacaagaccaacctgaagtctcatgagatgattcacacaggagaaatgccttatgtctgttccctatgtagccgtcgctttcgccaatcatccacttaccatcgtcacctgaggaattaccacagatctgactgaagtatctaacatcctcagcagagactggtagggcttcagcctcagtatgtcatcttcaaagagagaagaatgttgcaagtaaattgtactgtcccaataatgatataacatgcttgtggattgccacttttatgttttgttttttattgtgtgtgtgtgtgtatgtaattttttgtctgtaatttccatagttccacagcataagttattagaatactttgctgttaattcttgagttgcttcttgcttttagacagtgtctttctggttggcagctttatacacctgtctttctggcactagagtttccaaacattttctgatctccacttttattctctacagtggtcctgacagaggcctgccattccctctgacattttttaacatgttggggtttcatcccaagtcttagggttgcaagttaaatgcattgcctcttcagacatctcatgtcatgtctactgcttacagttcaagaatatttctctacattactagaatgacgttcaaagtggaataataaataaaaaaataatcaacaatt

SEQ ID NO: 5 - DNA, 1774 bp, Mus musculus
cacagtgcctccctgggcttcttggcatcaccattgaagttcactggagaaagaggtgaggtggagaagtaggtaaacttccctttcttgtggtcttgaatgtcttttacagtacatccgtcaactgttagcattttcctaaagtcacaaaacagatactaaactgctatagttgaatctttcagaccattgtcaccacaatggcttcacagcaggcaccagcaaaagaccttcagaccaacaatttagagtttactccaactgatagttctggtgtgcagtgggcagaagacatctctaactcaccaagtgctcagctaaacttttccccaagtaacaatggctgctgggcaactcaggagctgcaaagtctctggaagatgttcaactcctggttgcagccagaaaagcagactaaggagcagatgatttctcaactggtcttggagcagtttctcctcactgggcactgcaaggacaagtatgctttgacagagaagtggaaagccagtggtagcgatatgaggagattcatggagagtctgactgatgagtgcttgaagcctcctgtcatggtccatgtttcaatgcaaggacaagaagccctcttttctgaaaacatgccattaaaagaagtcatcaagcttttgaaacaacagcaatctgcaacaaggccaataccagataatgagcagatgccagtagacaccacacaagatagattattggccacaggcaagaaaacagtgaaaatgaatgcaacacctcttgcaatgctactgaagtaaatgttggtgaaagctgtagtggaaatgaaaaggactcccttcttattacccagaaagaacaaaaccatgagcatgaagaggggaatgttgtttgtcaattccctcgtggtgccagaagagcaagtcaagacacctccagtcatcatgtagacttcccgagtgctctgactcctgcagatgtccccatggaggaacaaccaatggatttatccagagaaaacatctctgaggacaagaacaattgctataacacttccaggaatgcagctactcaagtatataatggtgataatattcccaggaacaagacagactcccttttcattaacaagagaatatatcatcctgagcctgaggtgggagatattccttatggagttcctcaggattctacaagagcaagtcaaggaacatctacatgcctgcaagagtcacttggggaatgtttttctgaaaaagacccaagggaggtaccagggttgcagtctaggcaagagcagcctatctctgatcctgtccttggtaagaatcatgaggcaaacttaccatgtgaaagtcatcaaaagagattccatagagatgccaaactatacaagtgtgaagaatgttctaggatgttcaaacatgccaggagcctttcatcccaccagagaactcacctgaataagaagagtgaattgctttgcatcacctgtcagaaaatattcaaacgagtttctgaccttcgaacccatgagatcatacacatgtcagaaaagcctttcaagtgcagcacatgtgaaaagtccttcagccacaagaccaacctgaagtatcatgagatgattcacacaggagaaatgccttatgtctgttccctatgtagccgtcgctttcgccaatcatccacttaccatcgtcacctgaggaattaccacagatctgactgaagtatctaacatcctcagcagagactggtagggcttcagcctcagtatgtcatcttc

SEQ ID NO: 6 - DNA, 2273 bp, Mus musculus
cacagtgcctccctgggcttcttggcatcacccttgaagttcactggagaaagaggtgaggtggaggaataggtaaactttccttcctagtggtcttgaatgtcttttacagtacatccatcaactgttagcattttcgtaaagtcacaaaacagatattaaactactatagttgaatctttcacaccattgtcaccacaatggcttcacagcaggcaccagcaaaagaccttcagaccaacaatttagagtttactccaactgatagttctggtgtgcagtgggcagaagacatctctaactcaccaagtgctcagctaaacttttccccaagtaacaatggctgctgggcaactcaggagctgcaaagtctctggaagatgttcaactcctggttgcagccagaaaagcagactaaggagcagatgatttctcaactggtcttggagcagtttctcctcactgggcactgcaaggacaagtatgctttgactgagaagtggaaagccagtggtagcgatatgaggagattcatggagagtctgactgatgagtgcttgaagcctcctgtcatggtccatgtttcaatgcaaggacaagaagccctcttttctgaaaacatgccattaaaagaagtcatcaagcttttgaaacaacagcaatctgcaacaaggccaacaccagataatgagcagatgccagtagacaccacacaagatagattattggccacaggacaagaaaacagtgaaaatgaatgcaacaactcttgtaatgctactgaagcaaatgttggtgaaagctgtagtggaaatgaaatggactcccttcttattatgcagaaagaacagcaccctgagcatgaagaggggaatgttgtttgtcaattccctcatggtgccagaagagcaagtcaaggcacccccagtcatcatgtagacttcccgagtgctccgactactgccgatgtccccatggaggaacaaccaaaggatttatccagagaaaacatctctgaggacaagaacaattgctataacacttccagaaatgcagctactcaagtatatagtggtgataatattcccaggaacaagtcagactcccttttcattaacaagagaatatatcatcctgagcctgaggtgggagatattccttatggagttcctcaggattctacaagagcaagtcaaggaacatctacatgcctgcaagagtcacttggggaatgtttttctgaaaaagaccctagggaggtaccagggttgcagtctaggcaagagcagcttatctctgatcctgtccttcttggtaagaatcatgaggcaaacttaccatgtgaaagtcatcaaaagagattctgtagagatgccaaactatacaagtgtgaagaatgttctaggatgttcaaacatgccaggagcctttcatcccaccagagaactcacctgaataagaagagtgaattgctttgtgtcacctgtcagaaaatgttcaaacgagtctctgaccgccgaacccatgagatcatacacatgccagaaaagcctttcaagtgcagcacatgtgaaaagtccttcagccacaagaccaacctgaagtctcatgagatgattcacacaggagaaatgccttatgtctgttccctatgtagccgtcgctttcgccaatcatccacttaccatcgtcacctgaggaattaccacagatctgactgaactatctaacatcctcagcagagactggtagggcttcagcctcagtatgtcatcttcaaagagagaagaatgttgcaagtaaattgtactgtcccaataatgatataacatgcttgtggattgccacttttatgttttgttttgttttttattttgtgtgtgtgtgtatgtaattttttgtctgtatttccatagttccacagcataagttattagaatactttgctgttaattcttgagttgcttcttgcttttagacagtgtctttctggttgacagctttataaacctgtctttctggcactagagtttccaaacattttctgatctccacttttattctctacagtgttcttgacagaagcctggcattccctctgacatttttctacatgttggggttttcatcccaagtcttagggttgcaagttaaatgcattgcctcttcagacatctcatgccctgtctactgcttacagttcaagaatatttctctacattactagaacgacattcaaagtggaataataaataaataaataatcaacaatt

SEQ ID NO: 7 - DNA, 2260 bp, Homo sapiens
ccttgtaattcataaatctctgaaaacttaaaagtttgagcaaaagtttgtcatgtttctatgagtaatttataataaaacttgatcagaatttgtgagactaacgtttgtctttatattttccttttttttttttttttttttgagacacagtctcgctctgtcgtccaggctggagtgccgtggcgtaatctcggctcactgcaacctctgcctcctggattcaaacaattcttctgcctcagcctcctgagtagctgggattacaggaccagtgatggtatagaacactgtattagagacatggagctggggctggatgaagattccatcagtaattcaatcaacagacaagtgttatccaatcacgtctttaaatcaatcactgacatggagctggggctggatgaagattccatcagtaattcaatcaacagacaagtgttatccaatcacgtctttaaatcaatcactgatcccagcccctataaaagggagcagccttaggaggcacatcagataaacccagtgtggaaagctagtcacacatcagctcagtgttcggcccgggattacccagtcaaccaaggagcttgcagttttaaagaatccaccaactgttgaaacaaatccctagagacacaaggcaagagactgaatcatcaaagtaaagtctctctgagaattattgctaagaatggctttagatctaagaaccatatttcagtgtgaaccatccgagaataatcttggatcagaaaattcagcgtttcaacaaagccaaggacctgctgttcagagagaagaagggatttctgagttctcaagaatggtgctcaattcatttcaagacagcaataattcatatgcaaggcaggaattgcaaagactttataggatctttcactcatggctgcaaccagaaaagcacagcaaggatgaaattatttctctattagtcctggagcagtttatgattggtggccactgcaatgacaaagccagtgtgaaagagaaatggaaatcaagtggcaaaaacttggagagattcatagaagacctgactgatgacagcataaatccacctgccttagtccacgtccacatgcagggacaggaagctctcttttctgaggatatgcccttaagagatgtcattgttcatctcacaaaacaagtgaatgcccaaaccacaagagaagcaaacatggggacaccctcccagacttcccaagatacttccttagaaacaggacaaggatatgaagatgaacaagatggctggaacagttcttcgaaaactactcgagtaaatgaaaatattactaatcaaggcaatcaaatagtttccctaatcatcatccaggaagagaacggtcctaggcctgaagagggaggtgtttcttctgacaacccatacaactcaaaaagagcagagctagtcactgctagatctcaggaagggtccataaatggaatcactttccaaggtgtccctatggtgatgggagcagggtgtatctctcaaccagagcagtcctcccctgagtctgcccttacccaccagagcaatgagggaaattccacatgtgaggtacatcagaaaggatcccatggagtccaaaaatcatacaaatgtgaagaatgccccaaggtctttaagtatctctgtcacttattagctcaccagagaagacacaggaatgagaggccatttgtttgtcccgagtgtcaaaaaggcttcttccagatatcagacctacgggtgcatcagataattcacacaggaaagaagcctttcacatgcagcatgtgtaaaaagtccttcagccacaaaaccaacctgcggtctcatgagagaatccacacaggagaaaagccttatacatgtcccttttgtaagacaagctaccgccagtcatccacataccaccgccatatgaggactcatgagaaaattaccctgccaagtgttccctccacaccagaagcttcctaagctgctggtctgataatgtgtataaatatgtatgcaagtatgtatattcctatagtatttatctacttaggatataagatataatctcctgattatgctttcaatttattgtcttgcttcattaaaatgtaaggctaaggagagcatggaatttgtcagttttgttcactaaagtattccaagtggttgggaaagtggaacatttccaagaaccaataaatttctgttgaataaatgaatgaatccaaaaaaaaaaaaaaa

SEQ ID NO: 8 - DNA, 1302 bp, Canis familiaris
atggcttcagatatcagaatatcatttcagggagaaccatctatgaatgatcctgggtcagaaaacctagagcataaacttagccaaggaccagccattcaggaggaagacgagatctatgagttcccaagcactcagctcactttattgcaaaacagtaactcaagtgcaaggcaggaactgcaaaatctctataagttatttcactcatggctgcaaccagagaaacacagcaaggatgagattatttctcatctggtcttggaacagtttatgatcaatggccactgcagtgacaggtccatgttgaaaaagaaatggaatgcaagtggcaggaacctggagaaattcatggaagatctgactgatgatggcatgaagctacctggattagtccacgtccacatgaagggccaggacgccctcttttctgagaatatgcccttaagagaagtcatcgttcatttcatgaaacaattgtcagcaggaaccccaacagaagagaacatggggacaccctcctggacttcccaagatacttccctggaaacaggacaaggtgagtgggataaagcaaatggctacaacatttatcacaatgacggtactactagtcaaggcaatgcagtaccttccctgttcattgtccatgaggaggactgtcctcaccctgaagaggacagtgtttctttgaaggatctgctcagccctggaagaccgggtctaggtacgtccaattcccaggaagggtgcctgcaaggacgcccatatcaagatgtcctgatggagggggcaccagggtttcactctcggtcaaccgcagtcacccctgaccctgtttctacccaccaaaaaaccgaggggaattccacatgtgggggacaccaagaaagattccgtgacgcccaaaactcctacagatgtgaaaaatgtcccaggatctttaggtatttctctcagctaaaagcccatcagagaagacacaacaatgagaggacattcatttgtgctgagtgtaacaaaggcttcttccaagcgtcagacctacacgtgcatcagaagattcacacagaagagaagcctttcaggtgcagcacatgtgaaaaatccttcagccacaaaaccaaccttctggcccatgagagaatccacacgggtgagaagccctatgtatgtgcgctttgccagagaagctaccgccagtcatccacctaccaccgccacctgaggactcaccagaaaattgccgtcaaaggtactccttccacatcagaagcttcctcagctgtagcctcagtgtaa

SEQ ID NO: 9 - DNA, 1251 bp, Bos taurus
atggatttaggtttcagagcatcatttcagcatgaaccatccaatgaggacccaaagtcagcaaatacaggctttatccccagtcgaggacccactctgcaaacagcagaggatatctctcagttgcaaaacactcagcccggcttattgcaaaatggtaataactcacgtgcaaggcaggaactgcaaagactctataagtcatttcacttatggctgcagccagaaaaacacagcaagcatgaaattatttttcaacttgccctggaacaatttatgatcaataagcactgcagtgaaaagtctactttgaaagagaaatggaaagcaagtggtggagacctggagaaattcacagaagacctgcatgatgactgcataaagctacctgatttggtccatgtccacttgcaggggcaggaagccctcttttcagaaaatatgtccttaaaagaaatcatctttcatctaaccaatcagttgtcaacaggaggggtgaacatgggaactccgtcctggaccatgcaagatacatccctggaaacaggacaaagaaatgaaggtaaagaaaatgatggcaacatttctgtgaaaagtgacagtattactagtccaagcaatcagataccttccctaatcattgtccaagaagagaatcacctgaggctggaagaaggaggtgtttctctggagaatccacggaactccagaagaggagcaggcccaggcccctccaggcctcaggatggatccctgaaaggaccctcctctcaagatgtcctcatggaagtggaacgagaccaggtcacccctgggcctgtttctaccctccagagctctgaggggacttctgcacgtgggaaacaccaggaaagatccctcagagccccagaagtatacagatgtgagagatgtcccaagaccttcaggtattcctctcggttcagagttcaccagaaaagacacgataatgagagaacatatatttgtgccgagtgtggcaaaggcttctttcaggcctcagacctccatgtgcatcagaggattcatacaggagagaagccctttgtgtgcagcacatgtgaaatggccttcacccacaaaaccaaccttcgggctcacgagagaacccacacgggagagaagccctatgagtgttccctctgccagagacgcttccgccagtcctccacctaccaccgccatcttaggtttcaccagaaaactaccctcaaaagtgctccacactaa

SEQ ID NO: 10 - DNA, 1713 bp, Equus caballus
atggctttagatctcagaatctcatttcaaggtgaaccatccaggaatgatcctgggtcagaaaatcatgagtttaatccccgtcaagtacctgctgtccaggatggggagaggatctccaagttcccgagcactcaacacagcttatttcaaaatggcaagaattcatgtgcaaggcaggaactgcaaagactctataagttatttcactcctggctacagccagaaaaacacagcaaggatgaaatgatttctcgtttggtcctggagcaatttatgatcaatggctactgcagtgacaggtccatgttgaaagagaaatgggaatcaagtggcagaaacctggagaaattcatggaagatctgactgatgatggcatgaagccacctggcttagtccacgtctgcatgcaggggcaggaagctctcttttctgagaatatgcccttaagagaagtcatagttcacctcaggaaacagttctcaacaggaacccaaactggagagaacatggggacccctttccagactcccaaagatcattctctggaaacagaacaaggagatgaagacaaagaaaatggtggcaacatatctttgaaaacttgtcaagtaaatgacagtatgactagtcaaggcaatcaaacaccttccctactcatcatccagggagagaaccgtcctgggcctggagagggaggtgttcctttggagaatccactcagctccagaagagcaggtctaggcagctgcaggtcccaggaagagtccctgaaaggacccccttatcaagatgtccttatagaggtgagaccagggtttctctcccggccaaaccaggttacgcctgagcgtgttcctacccaccagagcattgagggaaactcagcatgtgggggacaccaagaaagatcccagggagcccccaaatcatacaaatgtgagaagtgtcccaggatctttaggtatctgtctcggttaaaagcccatcaaagaagacacaataatgagaggacatttatttgtggccagtgtgacaaaggcttcttccaggcatcagacctacgcatgcatcagaagattcacacaggagagaaacctttcaagtgcagcacatgtgaaatgtccttcagccacaaaaccaaccttcgggctcatgagagaatccacacaggggagaagccctatgtgtgttccctttgccagagaagctaccgccagtcatccacctaccaccgccacctgaggactcaccagaaaattgccttcaaaagtgttccctctagggggctgtggcagcataccagttcatggatccccacacagcagattcccacaactgtaagaggaggtgaggacagcatgaccggaaaacacttttgggctctggcccatgggagggcccaacatgccatagtggccttgcctgtggaaatgctctacactgagtggcggtggctcccctccaccctagcacagtgcaggcaagaaggtgccctgcccgctcagaaggtgcccctgtctgcagagcacagtagccagaaggatccacagagtggtggctcagcccccgcatgggtgccctacacccttagtgtagcgcaggcaagaaggcaccctgcccactcagaaggtaccccaacccacagagcatggcagcccacaggaaccatcaagtggcggctcagcctctacatagcctgcagcagctaa

SEQ ID NO: 11 - protein, 360 aa, Mus musculus
MASQQAPAKDLQTNNLEFTPTDSSGVQWAEDISNSPSAQLNFSPSNNGCWATQELQSLWKMFNSWLQPEKQTKEQMISQLVLEQFLLTGHCKDKYALTEKWKASGSDMRRFMESLTDECLKPPVMVHVSMQGQEALFSENMPLKEVIKLLKQQQSATRPTPDNAQMPVDTTQDRLLATGQENSENECNTSCNATEGNVGESCSGNEMDSSLIIQKEQYPEHEEGNVVCQFPLDARRASQGTSSHHVDFLSALTTADVPMEEQPKDLSRENISEDKNNCYNTSRNAATKVYSGDNIPRKKTDSLSINKRIYHPEPEVGDIPYGVPQDSTRASQGTSTCLQESLGGCFSEKDPREVPGLQSR

SEQ ID NO: 12 - protein, 195 aa, Mus musculus
MASQQAPAKDLQTNNLEFTPTDSSGVQWAEDISNSPSAQLNFSPSNNGCWATQELQSLWKMFNSWLQPEKQTKEQMISQLVLEQFLLTGHCKDKYALTEKWKASGSDMRRFMESLTDECLKPPVMVHVSMQGQEALFSENMPLKEVIKLLKQQQSATRPIPDNAQMPVDTTQDRLLATGKKTVKMNATPLAMLLK

SEQ ID NO: 13 - protein, 506 aa, Mus musculus
MASQQAPAKDLQTNNLEFTPTDSSGVQWAEDISNSPSAQLNFSPSNNGCWATQELQSLWKMFNSWLQPEKQTKEQMISQLVLEQFLLTGHCKDKYALTEKWKASGSDMRRFMESLTDECLKPPVMVHVSMQGQEALFSENMPLKEVIKLLKQQQSATRPTPDNEQMPVDTTQDRLLATGQENSENECNNSCNATEANVGESCSGNEMDSLLIIQKEQHPEHEEGNVVCQFPHGARRASQGTPSHHVDFPSAPTTADVPMEEQPKDLSRENISEDKNNCYNTSRNAATQVYSGDNIPRNKSDSLFINKRIYHPEPEVGDIPYGVPQDSTRASQGTSTCLQESLGECFSENDPREVPGLQSRQEQPISDPVLLGKNHEANLPCESHQKRFCRDAKLYKCEECSRMFKHARSLSSHQRTHLNKKSELLCVTCQKMFKRVSDRRTHEIIHMPEKPFKCSTCEKSFSHKTNLKSHEMIHTGEMPYVCSLCSRRFRQSSTYHRHLRNYHRSD

SEQ ID NO: 14 - protein, 506 aa, Mus musculus
MASQQAPAKDLQTNNLEFTPSHSSGVQWVEDISNSPSAQLNFSPSNNGCWATQELQSLWKMFNSWLQPEKQTKEQMISQLVLEQFLLIGHCKDKYALTEKWKASGSDMRRFMESLTDECLKPPVMVHVSMQGQEALFSENMPLKEVIKLLKQQQSATRPTPDNEQMPVDTTQDRLLATGQENSENECNNSCNATEANVGESCSGNEMDSLLIIQKEQHPEHEEGNVVFQFPLDARRASQGNSSHHVDFRSAPTPADVPMEEQPKDLSRENISEDKNNCYNTSRNAATQVYRSDNIPRKKTDSLSINKRIYHSEPEEGDIPYGVPQDSTRASQGTSTCLQESLGECFSEKDPRELPGLESRQEEPISDPVFLGKDHEANLPCESHQKRFRRDAKLFKCEECSRMFKHARSLSSHQRTHLNKKSELLCVTCQKMFKRVSDRRTHEIIHMPEKPFKCSTCEKSFSHKTNLKSHEMIHTGEMPYVCSLCSRRFRQSSTYHRHLRNYHRSD

SEQ ID NO: 15 - protein, 195 aa, Mus musculus
MASQQAPAKDLQTNNLEFTPTDSSGVQWAEDISNSPSAQLNFSPSNNGCWATQELQSLWKMFNSWLQPEKQTKEQMISQLVLEQFLLTGHCKDKYALTEKWKASGSDMRRFMESLTDECLKPPVMVHVSMQGQEALFSENMPLKEVIKLLKQQQSATRPIPDNEQMPVDTTQDRLLATGKKTVKMNATPLAMLLK

SEQ ID NO: 16 - protein, 506 aa, Mus musculus
MASQQAPAKDLQTNNLEFTPTDSSGVQWAEDISNSPSAQLNFSPSNNGCWATQELQSLWKMFNSWLQPEKQTKEQMISQLVLEQFLLTGHCKDKYALTEKWKASGSDMRRFMESLTDECLKPPVMVHVSMQGQEALFSENMPLKEVIKLLKQQQSATRPTPDNEQMPVDTTQDRLLATGQENSENECNNSCNATEANVGESCSGNEMDSLLIMQKEQHPEHEEGNVVCQFPHGARRASQGTPSHHVDFPSAPTTADVPMEEQPKDLSRENISEDKNNCYNTSRNAATQVYSGDNIPRNKSDSLFINKRIYHPEPEVGDIPYGVPQDSTRASQGTSTCLQESLGECFSEKDPREVPGLQSRQEQLISDPVLLGKNHEANLPCESHQKRFCRDAKLYKCEECSRMFKHARSLSSHQRTHLNKKSELLCVTCQKMFKRVSDRRTHEIIHMPEKPFKCSTCEKSFSHKTNLKSHEMIHTGEMPYVCSLCSRRFRQSSTYHRHLRNYHRSD

SEQ ID NO: 17 - protein, 433 aa, Homo sapiens
MALDLRTIFQCEPSENNLGSENSAFQQSQGPAVQREEGISEFSRMVLNSFQDSNNSYARQELQRLYRIFHSWLQPEKHSKDEIISLLVLEQFMIGGHCNDKASVKEKWKSSGKNLERFIEDLTDDSINPPALVHVHMQGQEALFSEDMPLRDVIVHLTKQVNAQTTREANMGTPSQTSQDTSLETGQGYEDEQDGWNSSSKTTRVNENITNQGNQIVSLIIIQEENGPRPEEGGVSSDNPYNSKRAELVTARSQEGSINGITFQGVPMVMGAGCISQPEQSSPESALTHQSNEGNSTCEVHQKGSHGVQKSYKCEECPKVFKYLCHLLAHQRRHRNERPFVCPECQKGFFQISDLRVHQIIHTGKKPFTCSMCKKSFSHKTNLRSHERIHTGEKPYTCPFCKTSYRQSSTYHRHMRTHEKITLPSVPSTPEAS

SEQ ID NO: 18 - protein, 433 aa, Canis familiaris
MASDIRISFQGEPSMNDPGSENLEHKLSQGPAIQEEDEIYEFPSTQLTLLQNSNSSARQELQNLYKLFHSWLQPEKHSKDEIISHLVLEQFMINGHCSDRSMLKKKWNASGRNLEKFMEDLTDDGMKLPGLVHVHMKGQDALFSENMPLREVIVHFMKQLSAGTPTEENMGTPSWTSQDTSLETGQGEWDKANGYNIYHNDGTTSQGNAVPSLFIVHEEDCPHPEEDSVSLKDLLSPGRPGLGTSNSQEGCLQGRPYQDVLMEGAPGFHSRSTAVTPDPVSTHQKTEGNSTCGGHQERFRDAQNSYRCEKCPRIFRYFSQLKAHQRRHNNERTFICAECNKGFFQASDLHVHQKIHTEEKPFRCSTCEKSFSHKTNLLAHERIHTGEKPYVCALCQRSYRQSSTYHRHLRTHQKIAVKGTPSTSEASSAVASV

SEQ ID NO: 19 - protein, 416 aa, Bos taurus
MDLGFRASFQHEPSNEDPKSANTGFIPSRGPTLQTAEDISQLQNTQPGLLQNGNNSRARQELQRLYKSFHLWLQPEKHSKHEIIFQLALEQFMINKHCSEKSTLKEKWKASGGDLEKFTEDLHDDCIKLPDLVHVHLQGQEALFSENMSLKEIIFHLTNQLSTGGVNMGTPSWTMQDTSLETGQRNEGKENDGNISVKSDSITSPSNQIPSLIIVQEENHLRLEEGGVSLENPRNSRRGAGPGPSRPQDGSLKGPSSQDVLMEVERDQVTPGPVSTLQSSEGTSARGKHQERSLRAPEVYRCERCPKTFRYSSRFRVHQKRHDNERTYICAECGKGFFQASDLHVHQRIHTGEKPFVCSTCEMAFTHKTNLRAHERTHTGEKPYECSLCQRRFRQSSTYHRHLRFHQKTTLKSAPH

SEQ ID NO: 20 - protein, 570 aa, Equus caballus
MALDLRISFQGEPSRNDPGSENHEFNPRQVPAVQDGERISKFPSTQHSLFQNGKNSCARQELQRLYKLFHSWLQPEKHSKDEMISRLVLEQFMINGYCSDRSMLKEKWESSGRNLEKFMEDLTDDGMKPPGLVHVCMQGQEALFSENMPLREVIVHLRKQFSTGTQTGENMGTPFQTPKDHSLETEQGDEDKENGGNISLKTCQVNDSMTSQGNQTPSLLIIQGENRPGPGEGGVPLENPLSSRRAGLGSCRSQEESLKGPPYQDVLIEVRPGFLSRPNQVTPERVPTHQSIEGNSACGGHQERSQGAPKSYKCEKCPRIFRYLSRLKAHQRRHNNERTFICGQCDKGFFQASDLRMHQKIHTGEKPFKCSTCEMSFSHKTNLRAHERIHTGEKPYVCSLCQRSYRQSSTYHRHLRTHQKIAFKSVPSRGLWQHTSSWIPTQQIPTTVRGGEDSMTGKHFWALAHGRAQHAIVALPVEMLYTEWRWLPSTLAQCRQEGALPAQKVPLSAEHSSQKDPQSGGSAPAWVPYTLSVAQARRHPAHSEGTPTHRAWQPTGTIKWRLSLYIACSS

SEQ ID NO: 21 - DNA, 528 bp, Gorilla gorilla
  misc_feature 18, 19, 80, 211, 212, 519, 520, 521, 522: n = A,T,C or G
aatggaatcactttccanngtgtccctatggtgatgggagcagggtgtatctctcaaccagagcagtcctcccctgagtntgcccttacccaccagagcaatgagggaaactccacatgtgaggtacatcagaaaggatcccatggagtccgaaaatcatacaaatgtgaagaatgccccaaggtctttaagtatcactgtcacttattanntcaccagagaagacacaggaatgagaggccatttgtttgtcccgagtgtcaaaaaggcttcttccagatatcagacctacgggtgcatcagataattcacacaggaaagaagcctttcacatgcagcatgtgtaaaaagtccttcagccacaaaaccaacctgcggtctcatgagagaatccacacaggagaaaagccttatacatgtcccttttgtaagacaagctaccgccagtcatccacataccaccgccatatgaggactcatgagaaaattaccctgccaagtgttccctccacaccagannnntcctaa

SEQ ID NO: 22 - DNA, 1302 bp, Pan paniscus
atggctttagatctaagaaccatatttcagtgtgaaccatccgagaataatcttggatcagaaaattcagcgtttcaacaaagccaaggacctgctgttcagagagaagaagggatttctgagttctcaagaatggtgctcaattcatttcaagacagcaataattcatatgcaaggcaggaattgcaaagactttataggatctttcactcatggctgcaaccagaaaagcacagcaaggatgaaattatttctctattagtcctggagcagtttatgattggtggccactgcaatgacaaagccggtgtgaaagagaaatggaaatcaagtggcaaaaacttggagagattcatagaagacctgactgatgacagcataaatccacctgccttagtccacgtccacatgcagggacaggaagctctcttttctgaggatatgcccttaagagatgtcattgttcatctcacaaaacaagtgaatgcccaaaccacaagagaagcaaacatggggacaccctcccagacttcccaagatacttccttagaaacaggacaaggatatgaagatgaacaagatggctggaacagttctttgaaaactactcaagtaaatgaaaatattactaatcaaggcgatcaaatagtttccctaatcatcatccaggaagagaacagtcctaggcctgaagagggaggtgtttcttctgacaacccatacaactcaaaaagagcagagctagtcactgctagatctcaggaagggtccataaatggaatcactttccaaggtgtccctatggtgatgggagcagggtgtatctctcaaccagagcagtcctcccctgagtctgcccttacccaccagagcaatgagggaaactccacatgtgaggtacatcagaaaggatcccatggagtccgaaaatcatacaaatgtgaagaatgccccaaggtctttaagtatctctgtcacttattagctcaccagagaagacacaggaatgagaggccatttgtttgtcccgagtgtcaaaaaggcttcttccagatatcagacctacgggtgcatcagataattcacacaggaaagaagcctttcacatgcagcatatgtaaaaagtccttcagccacaaaaccaacctgcggtctcatgagagaatccacacaggagaaaagccttatacatgtcccttttgtaagacaagctaccgccagtcatccacataccaccgccatatgaggactcatgagaaaattaccgtgccaagtgttccctccacaccagaagcttcctaa

SEQ ID NO: 23 - DNA, 1302 bp, Bornean orangutan
atggctttagatctaagaaccatatttcagtgtgaaccatccgagaataatcttggatcagaaaattcagagtttcgacaaagccaaggacctgctgttcagagagaagaagggatttctgagttctcaagaatggtgctcaattcatttcaagacagcaataattcatatgcaaggcaggaattgcagagactttataggatctttcactcatggctgcaaccagaaaagcacagcaaggatgaaattatttctctattagtcctggagcagtttatgattggtggccactgcaatgacaaagccagtgtgaaagagaaatggaaatcaagtggcaaaaacttggagagattcatggaagacctgactgatgacagcataaatccacctgccttagtccatgtccacatgcagggacaggaagctctcttttctgaggatatgcccttaaaagatgtcattgttcatctcacaaaacaagtgtctgcccaaaccccaagagaagcaaatatggggacaccctcccagacttcccaagatacttccttagaaacaggagaaggatgtgaagatgaacaagatggctgcaacagttctttgaaaactactcaagtaaatgaaaatattactaatcaaggcaatcaaatagtttccctaatcatcatccaggaagagaacggtcctaggtctgaagagggaggtgtttcttctgacaatccaaacaactcaaaaagagcagagctagtcactgctagatctcaggaagggtccataaacggaatcacttttcaaggtgtccctatggagatgggagcagggtgtatctctcagccagagcagtcctcccctgagtctgcccttacccaccagagcaatgagggaaactccacatgtgaggtacatcagaaaggatcccatggagtccgaaaatcctacaaatgtgaagaatgccctaaggtctttaagtatctctgtcacttattagctcaccagagaagacacaggaatgagaggccatttgtttgtcccgagtgtcaaaaaggcttcttccagatatcagacctacgcgtgcatcagataattcacacaggaaagaagcctttcacatgcagcatgtgtgaaaagtccttcagccacaaaaccaacctgcggtctcatgagagaatccacacaggagaaaagccttatacatgtcccttttgtaagacaagctaccgccagtcatccacataccaccgccatatgaggactcatgagaaaattaccccgccaagtgttccctccacaccagaagcttcctaa

SEQ ID NO: 24 - DNA, 1640 bp, Pongo abelii
tccaccaactgttgaaacaaatccctagagacacaaggcaagagactgaatcatcaaagtaaagtctctctgagaattattgctaagaatggctttagatctaagaaccatatttcagtgtgaaccatccgagaataatcttggatcagaaaattcagagtttcgacaaagccaaggacctgctgttcagagagaagaagggatttctgagttctcaagaatggtgctcaattcatttcaagacagcaataattcatatgcaaggcaggaattgcagagactttataggatctttcactcatggctgcaaccagaaaagcacagcaaggatgaaattatttctctattagtcctggagcagtttatgattggtggccactgcaatgacaaagccagtgtgaaagagaaatggaaatcaagtggcaaaaacttggagagattcatggaagacctgactgatgacagcataaatccacctgccttagtccatgtccacatgcagggacaggaagctctcttttctgaggatatgcccttaaaagatgtcattgttcatctcacaaaacaagtgtctgcccaaaccccaagagaagcaaatatggggacaccctcccagacttcccaagatacttccttagaaacaggagaaggatgtgaagatgaacaagatggctgcaacagttctttgaaaactactcaagtaaatgaaaatattactaatcaaggcaatcaaatagtttccctaatcatcatccaggaagagaacggtcctaggtctgaagagggaggtgtttcttctgacaatccaaacaactcaaaaagagcagagctagtcactgctagatctcaggaagggtccataaacggaatcacttttcaaggtgtccctatggagatgggagcagggtgtatctctcagccagagcagtcctcccctgagtctgcccttacccaccagagcaatgagggaaactccacatgtgaggtacatcagaaaggatcccatggagtccgaaaatcctacaaatgtgaagaatgccctaaggtctttaagtatctctgtcacttattagctcaccagagaagacacaggaatgagaggccatttgtttgtcccgagtgtcaaaaaggcttcttccagatatcagacctacgcgtgcatcagataattcacacaggaaagaagcctttcacatgcagcatgtgtgaaaagtccttcagccacaaaaccaacctgcggtctcatgagagaatccacacaggagaaaagccttatacatgtcccttttgtaagacaagctaccgccagtcatccacataccaccgccatatgaggactcatgagaaaattaccccgccaagtgttccctccacaccagaagcttcctaagctgctggtctgataatgtgtataaatatgtatgcaagtatgtatattcccatagtatttatcgacttaggatataagatataatttcctgattatgctttcaatttattgtcttgcttcattaaaatgtaaggctaaggagagcatggaatttgtcagttttgttcactaaagtattccaagtggttgggaaagtggaacatttccaagaaccaataaatttctgttgaataaatgaatgaatccaaaa

SEQ ID NO: 25 - DNA, 1002 bp, Artificial Sequence
  Reverse translation of SEQ ID NO: 35
ctgaaaattgatagctttctgtgcgaactgagcatggatgatccgggcagcaaaaacaaagattttaaaccgagccagggcccggcgctgcagaaagcggaagaaattagcgaatttcaggatagccagcatagcctgtttcaggatggcaacaacagccatgcgaaacaggaactgcagcgcctgtataaaagcttttatagctggctgcagccggaaaaacatagcaaagatgaaattatttttcaggtggtgctggaacagtttatgattaaccgccattgcagcggccgcagcaccctgaaaaaaaaatgggaaagcagcggccgcaacctggaaaaatttatggaaagcctgagcgaaagcagcctgaaaccgccggatctggtgcatgtgcatatgcagggccaggaagcgctgtttagcgaaaacatgccgctgaaagaagtgattgtgcatctgaccaaacagctgagcgtgggcagcccgaccggcaccgatatggaaaccccgagctggaccccgcaggataccagcctggaaaccggccagggcgaatggggcaaaaaagaaaacggcgataacatttatcatattaacgatagcattaccagccagggcaacgaaattccgagcctgctgattattcgcgaagaagattatccgcgcccggaagaagatagcgtgagcctgaaaaacccgctgagcagccgcaaagcgggcctgggcatgagcggcagccaggaaggcagcctgaaaggcccgagctatcaggatgtgctgatggaaggcggcccgggctttctgagccagagcattcaggtgagcccggaaccggtgccgacccatcagcgcaccgaaggcaacagcacccgcggcggccatcaggaacgctgccgcgaagcgcagaacagctatcgctgcgaaaaatgcccgaaaatttttcgctattttagccagctgaaagcgcatcagcgccgccataacaacgaacgcaccttt

SEQ ID NO: 26 - DNA, 1317 bp, Artificial Sequence
  Reverse translation of SEQ ID NO: 36
atggatctggatctgcgcctgagctttcagggcgaaccgagccgcaacgatccgggcagcgaaaacctggcgctgaaagcgagccagggctatgtgattcgcgatggcgaaggcattagcgaatttccgaacacccgcctgagcctgtttcagaacagcagcaacagctttgcgcgccgcgaactgcagcgcctgtataacctgtttcatagctggctgcagccggaaaaacgcagcaaagatgaaatgattagctgcctggtgctggaacagtttgtgattaacggccattgcagcgatcgcagcaccctgcaggaaaaatggaacgcgagcggccgcaacctggaaaaatttatggaagatctgaccgatgatggcatgaaacagccgggctttgtgcatgtgcatatgcagggccaggaagcgctgtttagcgaaaacatgccgctgcgcgaagtgctggtgcattttcgcaaacatctggcgaccgcgaccccgcgcggcgaaaacaccaaagcgccgctgtggaccccgcgcgatgcgagcctggaaaccggccaggaaagcgaaggcaaagaatgcggcggcaacaccagccgcaaaacctgcccggtgaccgaaagcctgacctggcagggcagccagaccccgtttctgctgattattccggaagaaacctgcccgggcctggaagaagcgggcgtgagcccggaaaacccgctgggcagccgcaccgcggaaccgggcctggcggtgagccaggaaggcagcccggaaggcccgtttggcggcgatgtgcatctggaagcggaaccgggctttctgagccgcccggatcaggtgaccctggaaccggtgagcgcgcatccgagcctggaaggcaacccggcgcgcggcaaaagcccggaaggcctgccgggcgcgcagaaagtgtttccgtgcgaaaaatgcagccaggtgtttcgctatctgagccgcctgaaagtgcatcagcgccgccataacgatgaacgcccgtttgtgtgcgcgaaatgcaaaaaaggcttttttcagaccagcgatctgcgcgtgcatcagcgcattcataccaaagaaaaaccgtttcgctgcagcacctgcaaacgcccgtttagccataaaaccaacctgcgcgcgcatgaacgcattcataccggcgaaaaaccgtatctgtgcagcctgtgccagcgccgctatcgccagagcagcacctataaccgccatctgaaaagccatcagaaactggcgctgaaaggcgatctgagcggcgtgccggtggtggcgcagcgcaaacgcatt

SEQ ID NO: 27 - DNA, 1656 bp, Nomascus leucogenys
agattgcagttttaaagaatccaccaactgttgaaacaaatccctagagacacaaggcaagagactgaatcatcaaagttaagtctctctgagaattattgctaagaatggctttagagctaagaaccatatttcagtgtgaaccatccgagaataatcttggatcagaaaattcagagtttcgacaaagccaaggacctgctgttcagagagaagaagggatttctgagttctcaagaatggtgctcaattcatttcaagacagcaataaatcatatgcaaggcaggaattgcaaagactttataggatctttcactcatggctgcaaccagaaaagcacagcaaggatgaaattatttctctattagtcctggagcagtttatgattggtggccactgcaatgacaaaaccagtgtgaaagagaaatggaaatcaagtggcaaaaacttggagagattcatggaagacctgactgatgacagcataaatccacctgccttagtccacgtccacatgcagggacaggaagctctcttttctgaggatatgcccttaaaagatgtcattgttcatctcacaaaacaagtgtctgcccaaatcccaagagaagcaaacatggggacacccttccagacttcccaagatacttccttagaaacaggacaaggacgtgaagatgaacaagatggctgcaacagttctttgaaaactactcaagtaaatgaaaatattactaatcaaggcaatcaaatagtttccctaatcatcatccaggaagagaatggtcctaggcctgaagagggaggtgtttcttctgacaacccatgcaactcaaaaagagcagagctagtcactgctagatcccaggaagggtccataaacggaatcacttttcaaggtgtccctatggagatgggagcagggtgtatctctcagccagagcagtcctcccctgagtctgcccctacccaccagagcaatgagggaaactccacatgtgaggtacatcagaaaggatcccatggagtccgaaaatcatacaaatgtgaagaatgccccaaggtctttaagtatctctgtcacttattagctcaccagaggagacacaggaatgagaggccatttgtttgtcccgagtgtcagaaaggcttcttccagacatcagacctacgcgtgcatcaggtgattcacacaggaaagaagcctttcacatgcagcatgtgtgaaaagtccttcagccacaaaaccaacctgcggtcccatgagagaatccacacaggagaaaagccttatacatgtccctattgtaagacaagctaccgccagtcatccacataccaccgccatatgaggactcatgagaaaattacctcaccaagtgttccctccacgccagaagcttcctaagctgctggtctgataatgtgtataaatgtgtatgcaagtatgtatattcccatagtatttatctacttaggatataagatataatttcctgattatgctttcaatttattgtctgcttcattaaaatgtaaggctaaggagagcatggaatttgtcagttttgctcactaaagtattccaagtggttgggaaagtgggaacatttccaagaaccaataaatttctgttgaataaatgaatgaatcca

SEQ ID NO: 28 - DNA, 1299 bp, Macaca mulatta
atggctttagatctaagaaccatatttcagcatgaaccatccgagaataatcttggatcagaaaattcagagtttcgacgaagtcaaggacctgctgttcagacagaagaagggatttctgagttctcaagaatgatgctcaattcatttcaagacagcaataattcatatgcaaggcaggaattgcaaagactttataggatctttcactcatggctgcaaccagaaaagcacagcaaggatgaaattatttctctattagtcctggagcagtttatgattggtggccactgcaatgacaaagccactgtgaaagagaaatggaaatcaagtggcaaaaacctggagagattcatggaagacctgactgatgacatcataaatccacctgccttagtccatgtccacatgcagggacaggaagctctcttttctgacaatatgcccttaaaagatgtcattgttcatctcacaaaacaagtgtctgccaaaactccaagagaagcaaacatggggacacccttccagacttcccaagacacttcctcagaaacaggacaaggacgtgaagatgaacaagatggctgcaacagttctttgaaaactactcaagtaaatgaaagtaatactaatcaagacaatccaatagtttctctaatcatccaggaagagaatggccctaggcctaaagagggaggtgtttcttctgacaacccatacaattcaagaagaacagagctagacactgctagatcccaggaagggtccacgaacggaattatttttcaaggtgtccctatggagatgggagcagggtttatctctcagccagagcagtcatcccctgagtctgcccctacccaccagagcaataaggggaactccacatgtgaggtacatcagaaaggatcccatggagtccgaaaatcatacaaatgtgaagaatgccccaaggtctttaagtatctctgtcacttattagctcaccagagaagacacaggaatgagaggccatttgtttgtcccaagtgtcaaaaaggcttcttccagatatcagacctacgtgtgcatcagataattcacacaggagagaaaccttttacatgcagcatgtgtgaaaagtccttcagccacaaaaccaacctgcggtctcatgagagaatccacacaggagaaaagccttatacatgtccctattgtaagagaagctaccgccagtcatccacataccaccgccatatgaggactcataagaaaattactctgccaactgttccctccacaccagaagcttcctaa

SEQ ID NO: 29 - DNA, 1008 bp, Artificial Sequence
  Reverse translation of SEQ ID NO: 39
atggcgctggatctgcgcaaaagcttttgccaggaactgagcagcaacaacctggaaagcgaagatctggaatttagcagcacccagggctttgcggtgccgaaacgcgaaattagcgcgtttagcagcattcagctgaacagcctgcagtatagcgataacagcgaagcgcgcaaagaactgcagcgcctgtatgaattttttcatagctggctgcagccggaaaaccatagcaaagatcagattattgcgcagctggcgatggaacagtttatgctgagcggccgctgccgcgataaaagcattctgaaaaaaaaatgggaaagcagcggcaaaaacctggaaaaactgctggaagatctgaccgatgattgcatgaaaccgccggtgctggtgcatgtgtgcatgcagggccaggaagcgctgtttagcgaagatatgccgctgaaagaagtgattgcgcatctgaccaaacagagcagcgcgaaaacctttaccgcgggcatgggcaccgcgcatcaggtgagccagaacgcgccgctgggcacccgccagggcaacgaacatgaagaagatggctgcaccagcagctgggaagtgacccaggtgaacgattatattaccaacccgggcaaagaaattgtgagcctgctgattattccggaagcgaacgatccgaccccggtggaagaaagcgcgagctgggaaaacacccatagcagccgcaaagcgcgcccggtgatttgcggcctgcaggaagaaagccagaaaggcccgagctatcaggatgtgccgatggatgtgggcccgggcagcagcagcctgccgcatcagagcagcagcgaaccggtgagcaaccatcattgcagcgaaggcaacagcgcgtgcgaagaaagccaggaacgctttcatgaaagcccgaaaagctataaatgcgaagaatgcccgaaaacctttaaatatctgagccattttctggcgcatcagcgctgccatcgcagctttcgc

SEQ ID NO: 30 - DNA, 990 bp, Artificial Sequence
  Reverse translation of SEQ ID NO: 40
atgccgagcaacctgaccaacagctgccagtgcaaaaccagccagaacgattttgaactgggcaacaccgaatttcgccgcacccagggcagcgcggtgcagaacggcgaaatttttagcgaatttagcagcagccagctgaacagcctgccggataacggcaacagcaacgcgcgcaaagaactgcagcgcctgcatggcatttttcatagctggctgcagccggaaaaacatagcaaagatgaaattattagccgcctggtgctggaacagtttatgattaacggcaactgccgcgatcgcagcattctgaaagaaaaatgggaaagcagcggccgcaacctggaaaaactgatggaagatctgaccgatgattgcatggaaccgccggtgctggtgcgcgtgcatatgcagggccaggaagcgctgtttagcgaaaacatgccgctgaaagaagtgattgtgcatctgaaaaaacagctgagcgcggaaaacaccaccggcgaaaacaaaggcatgagcctgcaggcgccgcaggataccccgctggaaacccgccagggcaacgaagataaagaaaacgcgtgcaacaacttttggaaaaacacccaggtggatgatagcattacctgccagggcacccagaccccgagcctgctgattattcaggaagatcattgcctgcgcctggaagatggcggcgcgagctgcgaaaacccgcataacagccgccgcggcgtgaccagccatagcgaaaaaggcccgctggaaggcccgagctatcagaacattccggtgggcgaacagccggaatttctgccgaccagcgatcagagcagcagcgaatttgtgccggcgcatcagagcaacaaaggcgatagcacctgcggcggccatcatgaaaaatatcgcggcgcgcagaaaagctataaatgcaaagaatgcccgaaaatttttcgctatctgtgccattttctggcgcatcagcgc

SEQ ID NO: 31 - protein, 175 aa, Gorilla gorilla
  VARIANT 6, 7, 27, 71, 173, 174: Xaa = Any Amino Acid
NGITFXXVPMVMGAGCISQPEQSSPEXALTHQSNEGNSTCEVHQKGSHGVRKSYKCEECPKVFKYHCHLLXHQRRHRNERPFVCPECQKGFFQISDLRVHQIIHTGKKPFTCSMCKKSFSHKTNLRSHERIHTGEKPYTCPFCKTSYRQSSTYHRHMRTHEKITLPSVPSTPXXS

SEQ ID NO: 32 - protein, 433 aa, Pan paniscus
MALDLRTIFQCEPSENNLGSENSAFQQSQGPAVQREEGISEFSRMVLNSFQDSNNSYARQELQRLYRIFHSWLQPEKHSKDEIISLLVLEQFMIGGHCNDKAGVKEKWKSSGKNLERFIEDLTDDSINPPALVHVHMQGQEALFSEDMPLRDVIVHLTKQVNAQTTREANMGTPSQTSQDTSLETGQGYEDEQDGWNSSLKTTQVNENITNQGDQIVSLIIIQEENSPRPEEGGVSSDNPYNSKRAELVTARSQEGSINGITFQGVPMVMGAGCISQPEQSSPESALTHQSNEGNSTCEVHQKGSHGVRKSYKCEECPKVFKYLCHLLAHQRRHRNERPFVCPECQKGFFQISDLRVHQIIHTGKKPFTCSICKKSFSHKTNLRSHERIHTGEKPYTCPFCKTSYRQSSTYHRHMRTHEKITVPSVPSTPEAS

SEQ ID NO: 33 - protein, 433 aa, Pongo pygmaeus
MALDLRTIFQCEPSENNLGSENSEFRQSQGPAVQREEGISEFSRMVLNSFQDSNNSYARQELQRLYRIFHSWLQPEKHSKDEIISLLVLEQFMIGGHCNDKASVKEKWKSSGKNLERFMEDLTDDSINPPALVHVHMQGQEALFSEDMPLKDVIVHLTKQVSAQTPREANMGTPSQTSQDTSLETGEGCEDEQDGCNSSLKTTQVNENITNQGNQIVSLIIIQEENGPRSEEGGVSSDNPNNSKRAELVTARSQEGSINGITFQGVPMEMGAGCISQPEQSSPESALTHQSNEGNSTCEVHQKGSHGVRKSYKCEECPKVFKYLCHLLAHQRRHRNERPFVCPECQKGFFQISDLRVHQIIHTGKKPFTCSMCEKSFSHKTNLRSHERIHTGEKPYTCPFCKTSYRQSSTYHRHMRTHEKITPPSVPSTPEAS

SEQ ID NO: 34 - protein, 433 aa, Pongo abelii; identical to SEQ ID NO: 33

SEQ ID NO: 35 - protein, 334 aa, Ailuropoda melanoleuca
LKIDSFLCELSMDDPGSKNKDFKPSQGPALQKAEEISEFQDSQHSLFQDGNNSHAKQELQRLYKSFYSWLQPEKHSKDEIIFQVVLEQFMINRHCSGRSTLKKKWESSGRNLEKFMESLSESSLKPPDLVHVHMQGQEALFSENMPLKEVIVHLTKQLSVGSPTGTDMETPSWTPQDTSLETGQGEWGKKENGDNIYHINDSITSQGNEIPSLLIIREEDYPRPEEDSVSLKNPLSSRKAGLGMSGSQEGSLKGPSYQDVLMEGGPGFLSQSIQVSPEPVPTHQRTEGNSTRGGHQERCREAQNSYRCEKCPKIFRYFSQLKAHQRRHNNERTF

SEQ ID NO: 36 - protein, 439 aa, Sus scrofa
MDLDLRLSFQGEPSRNDPGSENLALKASQGYVIRDGEGISEFPNTRLSLFQNSSNSFARRELQRLYNLFHSWLQPEKRSKDEMISCLVLEQFVINGHCSDRSTLQEKWNASGRNLEKFMEDLTDDGMKQPGFVHVHMQGQEALFSENMPLREVLVHFRKHLATATPRGENTKAPLWTPRDASLETGQESEGKECGGNTSRKTCPVTESLTWQGSQTPFLLIIPEETCPGLEEAGVSPENPLGSRTAEPGLAVSQEGSPEGPFGGDVHLEAEPGFLSRPDQVTLEPVSAHPSLEGNPARGKSPEGLPGAQKVFPCEKCSQVFRYLSRLKVHQRRHNDERPFVCAKCKKGFFQTSDLRVHQRIHTKEKPFRCSTCKRPFSHKTNLRAHERIHTGEKPYLCSLCQRRYRQSSTYNRHLKSHQKLALKGDLSGVPVVAQRKRI

SEQ ID NO: 37 - protein, 433 aa, Nomascus leucogenys
MALELRTIFQCEPSENNLGSENSEFRQSQGPAVQREEGISEFSRMVLNSFQDSNKSYARQELQRLYRIFHSWLQPEKHSKDEIISLLVLEQFMIGGHCNDKTSVKEKWKSSGKNLERFMEDLTDDSINPPALVHVHMQGQEALFSEDMPLKDVIVHLTKQVSAQIPREANMGTPFQTSQDTSLETGQGREDEQDGCNSSLKTTQVNENITNQGNQIVSLIIIQEENGPRPEEGGVSSDNPCNSKRAELVTARSQEGSINGITFQGVPMEMGAGCISQPEQSSPESAPTHQSNEGNSTCEVHQKGSHGVRKSYKCEECPKVFKYLCHLLAHQRRHRNERPFVCPECQKGFFQTSDLRVHQVIHTGKKPFTCSMCEKSFSHKTNLRSHERIHTGEKPYTCPYCKTSYRQSSTYHRHMRTHEKITSPSVPSTPEAS

SEQ ID NO: 38 - protein, 432 aa, Macaca mulatta
MALDLRTIFQHEPSENNLGSENSEFRRSQGPAVQTEEGISEFSRMMLNSFQDSNNSYARQELQRLYRIFHSWLQPEKHSKDEIISLLVLEQFMIGGHCNDKATVKEKWKSSGKNLERFMEDLTDDIINPPALVHVHMQGQEALFSDNMPLKDVIVHLTKQVSAKTPREANMGTPFQTSQDTSSETGQGREDEQDGCNSSLKTTQVNESNTNQDNPIVSLIIQEENGPRPKEGGVSSDNPYNSRRTELDTARSQEGSTNGIIFQGVPMEMGAGFISQPEQSSPESAPTHQSNKGNSTCEVHQKGSHGVRKSYKCEECPKVFKYLCHLLAHQRRHRNERPFVCPKCQKGFFQISDLRVHQIIHTGEKPFTCSMCEKSFSHKTNLRSHERIHTGEKPYTCPYCKRSYRQSSTYHRHMRTHKKITLPTVPSTPEAS

SEQ ID NO: 39 - protein, 336 aa, Cavia porcellus
MALDLRKSFCQELSSNNLESEDLEFSSTQGFAVPKREISAFSSIQLNSLQYSDNSEARKELQRLYEFFHSWLQPENHSKDQIIAQLAMEQFMLSGRCRDKSILKKKWESSGKNLEKLLEDLTDDCMKPPVLVHVCMQGQEALFSEDMPLKEVIAHLTKQSSAKTFTAGMGTAHQVSQNAPLGTRQGNEHEEDGCTSSWEVTQVNDYITNPGKEIVSLLIIPEANDPTPVEESASWENTHSSRKARPVICGLQEESQKGPSYQDVPMDVGPGSSSLPHQSSSEPVSNHHCSEGNSACEESQERFHESPKSYKCEECPKTFKYLSHFLAHQRCHRSFR

SEQ ID NO: 40 - protein, 330 aa, Spermophilus tridecemlineatus
MPSNLTNSCQCKTSQNDFELGNTEFRRTQGSAVQNGEIFSEFSSSQLNSLPDNGNSNARKELQRLHGIFHSWLQPEKHSKDEIISRLVLEQFMINGNCRDRSILKEKWESSGRNLEKLMEDLTDDCMEPPVLVRVHMQGQEALFSENMPLKEVIVHLKKQLSAENTTGENKGMSLQAPQDTPLETRQGNEDKENACNNFWKNTQVDDSITCQGTQTPSLLIIQEDHCLRLEDGGASCENPHNSRRGVTSHSEKGPLEGPSYQNIPVGEQPEFLPTSDQSSSEFVPAHQSNKGDSTCGGHHEKYRGAQKSYKCKECPKIFRYLCHFLAHQR

SEQ ID NO: 41 - DNA, 39 bp, Artificial Sequence
  Synthetic Construct
cggtttgtttgggtttgggtttgggtttgggtttgggtt

SEQ ID NO: 42 - DNA, 39 bp, Artificial Sequence
  Synthetic Construct
ggcttgccttacccttacccttacccttacccttaccct

SEQ ID NO: 43 - DNA, 23 bp, Artificial Sequence
  Synthetic Construct
cagcaagtgggaaggtgtaatcc

SEQ ID NO: 44 - DNA, 25 bp, Artificial Sequence
  Synthetic Construct
cccattctatcatcaacgggtacaa